European Patent Specification EP 3 076 918 B1, published August 5, 2026. Title: LIPOSOMAL PARTICLES, METHODS OF MAKING SAME AND USES THEREOF. Applicant: Northwestern University Mirkin, et al. The sequence listing filed with the application follows.

SEQUENCE LISTING (8 sequences)

SEQ ID NO: 1 - DNA, 25 bp, Artificial Sequence
  Synthetic polynucleotide
ttttttttttttttttttttttttt

SEQ ID NO: 2 - DNA, 19 bp, Artificial Sequence
  Synthetic polynucleotide
aaaaaaaaaatctcttgga

SEQ ID NO: 3 - DNA, 19 bp, Artificial Sequence
  Synthetic polynucleotide
tgcgtagacaaaaaaaaaa

SEQ ID NO: 4 - DNA, 18 bp, Artificial Sequence
  Synthetic polynucleotide
acgcatctgtccaagaga

SEQ ID NO: 5 - DNA, 25 bp, Artificial Sequence
  Synthetic polynucleotide
ctccatggtgctcactttttttttt

SEQ ID NO: 6 - DNA, 25 bp, Artificial Sequence
  Synthetic polynucleotide
ctccatggtgctcactttttttttt

SEQ ID NO: 7 - DNA, 29 bp, Artificial Sequence
  Synthetic polynucleotide
gagctgcacgctgccgtcatttttttttt

SEQ ID NO: 8 - DNA, 24 bp, Artificial Sequence
  Synthetic polynucleotide
tcgtcgttttgtcgttttgtcgtt